European Patent Specification EP 3 943 092 B1, published November 13, 2024. Title: Methods and Compositions for Inducing Differentiation of Human Brown Adipocyte Progenitors. Applicant: Energesis Pharmaceuticals, Inc. Application US 15/120,850. The sequence listing filed with the application follows.

SEQUENCE LISTING (9 sequences)

SEQ ID NO: 1 - DNA, 20 bp, Artificial Sequence
  Synthetic
tcaaggggttggtaccttcc

SEQ ID NO: 2 - DNA, 20 bp, Artificial Sequence
  Synthetic
cactaacgaaggaccaacgg

SEQ ID NO: 3 - DNA, 20 bp, Artificial Sequence
  Synthetic
ttccaggatccaagtcgcaa

SEQ ID NO: 4 - DNA, 20 bp, Artificial Sequence
  Synthetic
actgccaagactgagtggtt

SEQ ID NO: 5 - DNA, 20 bp, Artificial Sequence
  Synthetic
caaatgctggacccaacaca

SEQ ID NO: 6 - DNA, 20 bp, Artificial Sequence
  Synthetic
tcactttgccaaacaccaca

SEQ ID NO: 7 - DNA, 22 bp, Artificial Sequence
  Synthetic
tcacaagaaatgaccatggttg

SEQ ID NO: 8 - DNA, 22 bp, Artificial Sequence
  Synthetic
agcgattccttcactgatacac

SEQ ID NO: 9 - DNA, 20 bp, Artificial Sequence
  Synthetic
ccagaatggcatctctgtgt